European Patent Application EP 4 814 120 A1, published September 30, 2026. Title: Microorganisms and a method for producing L-amino acids using the same. Applicant: CJ CheilJedang Corporation. Application KR. The sequence listing filed with the application follows.

SEQUENCE LISTING (146 sequences)

SEQ ID NO: 1 - protein, 469 aa, Corynebacterium glutamicum
MTEQEFRIEHDTMGEVKVPAKALWQAQTQRAVENFPISGRGLESAQIRAMGLLKAACAQVNKDSGALDAEKADAIIAAGKEIASGKHDAEFPIDVFQTGSGTSSNMNTNEVIASIAKANGVEVHPNDHVNMGQSSNDTFPTATHVAATEAAVNDLIPGLKVLHESLAKKANEWSEVVKSGRTHLMDAVPVTLGQEFGGYARQIQLGIERVEATLPRLGELAIGGTAAGTGINTSADFGGKVVAELINLTDVKELKEAENHFEAQAARDALVEFSGAMRVIAVSLYKIANDIRLMGSGPLTGLGEIRLPDLQPGSSIMPGKVNPVLCETATQVSAQVIGNDAAVAFSGTQGQFELNVFIPVMARNVLESARLLANTSRVFATRLVDGIEPNEAHMKELAESSPSIVTPLNSAIGYEAAAKVAKTALAEGKTIRQTVIDLGLVDGEKLTEEELDKRLDVLAMAHTERENKF

SEQ ID NO: 2 - DNA, 1410 bp, Corynebacterium glutamicum
  source 1..1410: mol_type = genomic DNA
atgaccgagcaggaattccgtattgagcacgacaccatgggtgaagtgaaggttccagcaaaggctctgtggcaggcacagacccagcgcgctgttgagaacttccctatctctggtcgtggtctggaatccgcacagatccgcgcaatgggtctgctgaaggcagcttgtgcgcaggtaaacaaggactccggtgcgctggatgcagagaaggcagatgccatcattgcagctggtaaggagatcgcgtccggtaagcatgacgctgagttcccaattgatgtgttccagactggttccggtacttcctccaacatgaacaccaatgaggttatcgcttccatcgcgaaggctaacggcgttgaggttcacccaaatgaccacgtcaacatgggtcagtcctccaatgacaccttccctactgcaactcacgttgctgcaaccgaagctgctgtcaatgacctcatcccaggcctgaaagttctgcacgagtctttggcgaagaaggctaacgagtggtctgaggttgttaagtccggccgcacccacctgatggacgctgttccagtaaccctgggccaggagttcggtggctacgctcgccagatccagctcggcatcgagcgcgttgaggctactcttcctcgccttggtgagctggctattggtggcaccgctgctggtaccggtatcaacacctccgctgatttcggcggcaaggttgttgctgaactgatcaacttgaccgacgtcaaggagctcaaggaagctgagaaccacttcgaggctcaggctgcacgcgacgctcttgttgagttctccggcgcaatgcgcgttatcgctgtctccttgtacaagatcgctaacgatatccgcctcatgggctccggcccactgaccggtcttggcgagatccgtctcccagacctgcagccgggttcctccatcatgccaggcaaggtcaacccagttctctgtgagaccgctacccaggtttccgctcaggttatcggcaatgacgcagctgttgcgttctccggcacccagggccagttcgagctcaacgtgttcatcccagtgatggctcgcaacgtgcttgagtccgctcgcctgctggctaacacttcccgcgtgttcgcaacccgtctcgttgatggcattgagccaaacgaggcacacatgaaggagctcgctgagtcttcaccttccatcgttaccccactgaactctgcaatcggctacgaagctgctgcaaaggtggctaagactgctttggctgagggcaagaccatccgccagactgtcatcgatttgggcttggttgatggcgagaagctcaccgaggaagagctggacaagcgcctcgacgttcttgctatggctcacaccgagcgcgagaacaagttctaa

SEQ ID NO: 3 - protein, 401 aa, Corynebacterium glutamicum
MGPYYGPRTLHQVLREDYTTLFNELSSLGLPAQVCGALLHLTQRPSLRFSYMSCVVPLFADEIKVVGQGTRLSLEEKMMIQRFHDTGVSAAEIGRRLGRCRQTISRELRRGQDDDGCYRARDSYEGAIRKLARPKTPKLDANRRLRAVVVEALNKKLSPEQISGLLATEHANDSSMQISHETIYQALYVQGKGALRDELKVEKFLRTGRKGRKPQSKLPSRGKPWVEGALISQRPAEVDDRAVPGHWEGDLVIGGENQATALVTLVERTSRLTLIKRLGVNHEASTVTDALVEMMGDLPQALRRSLTWDQGVEMAEHARFSVVTKCPVFFCDPHSPWQRGSNENTNGLVRDFFPKGTNFAKVSDEEVQRAQDLLNYRPRKMHGFKSAAQVYEKIVVGASTD

SEQ ID NO: 4 - DNA, 1206 bp, Corynebacterium glutamicum
  source 1..1206: mol_type = genomic DNA
atgggcccttattatgggccacgcacactgcatcaagtattgcgtgaggactacacaacactgtttaacgagttgtcctcgttggggctgccggcacaggtgtgtggggccttacttcatctcacgcaacgaccatcattacgcttttcttatatgtcgtgtgtggtgccgttatttgctgatgaaatcaaagtcgtaggacaaggcacacgattatcgctagaagagaaaatgatgatccaacgcttccatgacaccggggtcagtgcagcagaaatcggtcgacgtctgggtcggtgtcggcaaacaatttcccgggaacttcgtcgtggtcaagatgatgacgggtgttatcgtgcacgcgactcctatgagggtgcgattaggaaactagcacgtccgaaaactccgaaacttgatgccaatcgtaggcttcgggctgtggtggtcgaggcgctgaataaaaaattatctccggagcagatttctggccttttagccactgagcatgctaacgatagctctatgcagattagtcatgaaactatttaccaggcgttatatgttcagggtaaaggggcgttgcgtgatgagttgaaggtggagaagtttcttcgtaccggtcggaagggacgtaaaccgcagtcgaagttgccatcgagaggtaaaccgtgggtggagggtgcgttgattagtcaacgcccggctgaggttgatgatcgtgctgtgcctgggcactgggagggcgatttggttattggtggtgaaaaccaagccacggcgttggtgacgttggtggagcggacaagtcggttgacgttgattaagcggttgggtgttaatcatgaggcgtcgactgtgacggatgcgttggtggagatgatgggtgatttgccgcaggcgttgcgtcggagtttgacgtgggatcagggtgtggagatggcagagcatgcgcggtttagtgtggtgaccaagtgtccggtgtttttctgtgatcctcattcgccgtggcagcgtgggtcgaatgagaatacgaatggattggtcagggattttttcccgaagggcactaattttgctaaagtaagtgacgaagaagttcagcgggcacaggatctgctgaattaccggccgcggaagatgcatggttttaaaagcgcggctcaggtgtatgaaaaaatcgtagttggtgcatccaccgattga

SEQ ID NO: 5 - DNA, 40 bp, synthetic construct
  source 1..40: mol_type = other DNA
aaacgacggccagtgaattctggccataacgagtgcggta

SEQ ID NO: 6 - DNA, 45 bp, synthetic construct
  source 1..45: mol_type = other DNA
ggctcttcctgtttagtactaaaccggaacccgggccttcacccc

SEQ ID NO: 7 - DNA, 43 bp, synthetic construct
  source 1..43: mol_type = other DNA
gacggattcagggggtgaaggcccgggttccggtttagtacta

SEQ ID NO: 8 - DNA, 40 bp, synthetic construct
  source 1..40: mol_type = other DNA
cttgcatgcctgcaggtcgactgctggagtgagcgcatga

SEQ ID NO: 9 - DNA, 294 bp, synthetic construct
  source 1..294: mol_type = other DNA
ggcgcttcatgtcaacaatctttaacgttttcaagttcacaagtcgtgttcaaatggtgacaagattggacactgtgctgaattggcaccaagccctcataaatgatagatctaaatcgaatatcaatatatggtctgtttattggaacgcgtcccagtggctgagacgcatccgctaaagccccaggaaccctgtgcagaaagaacaaataatcgtgaattttggcagcaacagcggggcctggtataattgaaaacgtgcaaaagcatagattattggaggagatcaaaaca

SEQ ID NO: 10 - DNA, 42 bp, synthetic construct
  source 1..42: mol_type = other DNA
gattattggaggagatcaaaacaatgaccgagcaggaattcc

SEQ ID NO: 11 - DNA, 37 bp, synthetic construct
  source 1..37: mol_type = other DNA
ggctcttcctgtttagtttagaacttgttctcgcgct

SEQ ID NO: 12 - DNA, 43 bp, synthetic construct
  source 1..43: mol_type = other DNA
ggcccttccggtttagtggcgcttcatgtcaacaatctttaac

SEQ ID NO: 13 - DNA, 42 bp, synthetic construct
  source 1..42: mol_type = other DNA
ggaattcctgctcggtcattgttttgatctcctccaataatc

SEQ ID NO: 14 - DNA, 40 bp, synthetic construct
  source 1..40: mol_type = other DNA
tgaattcgagctcggtaccccactggtgaactccttgtcc

SEQ ID NO: 15 - DNA, 40 bp, synthetic construct
  source 1..40: mol_type = other DNA
ttgaactaggggcgctttaaaagttttccggtgttgacgg

SEQ ID NO: 16 - DNA, 40 bp, synthetic construct
  source 1..40: mol_type = other DNA
ccgtcaacaccggaaaacttttaaagcgcccctagttcaa

SEQ ID NO: 17 - DNA, 40 bp, synthetic construct
  source 1..40: mol_type = other DNA
gtcgactctagaggatcccccgttgaactgcttgccagcc

SEQ ID NO: 18 - DNA, 40 bp, synthetic construct
  source 1..40: mol_type = other DNA
tgaattcgagctcggtaccctgcggctcgcacggttgctc

SEQ ID NO: 19 - DNA, 40 bp, synthetic construct
  source 1..40: mol_type = other DNA
acggtgcgcaagaagaccacgtcggcagcaaaagcagcct

SEQ ID NO: 20 - DNA, 40 bp, synthetic construct
  source 1..40: mol_type = other DNA
ggctgcttttgctgccgacgtggtcttcttgcgcaccgtg

SEQ ID NO: 21 - DNA, 40 bp, synthetic construct
  source 1..40: mol_type = other DNA
gtcgactctagaggatccccctcttatcaggccaatcggt

SEQ ID NO: 22 - protein, 347 aa, Corynebacterium glutamicum
MIIKVAIAGASGYAGGEILRLLLGHPAYASGELEIGALTAASTAGSTLGELMPHIPQLADRVIQDTTAETLAGHDVVFLGLPHGFSAEIALQLGPDVTVIDCAADFRLQNAADWEKFYGSEHQGTWPYGIPEIPGHREALRGAKRVAVPGCFPTGATLALLPAVQAGLIEPDVSVVSITGVSGAGKKASVALLGSETMGSLKTYNTSGKHRHTPEIAQNLGEVSDKPVKVSFTPVLAPLPRGILTTATAPLKEGVTAEQARAVYEEFYAQETFVHVLPEGAQPQTQAVLGSNMCHVQVEIDEEAGKVLVTSAIDNLTKGTAGAAVQCMNLSVGFDEAAGLPQVGVAP

SEQ ID NO: 23 - DNA, 1044 bp, Corynebacterium glutamicum
  source 1..1044: mol_type = genomic DNA
atgataatcaaggttgcaatcgcaggagccagtggatatgccggcggagaaatccttcgtctccttttaggccatccagcttatgcatctggtgaactagaaatcggagcactcaccgcggcatcaaccgcaggcagcacgctcggtgaattgatgccacacattccgcagttggcggatcgtgttattcaagacaccacagctgaaactctagccggtcatgatgtcgtatttctaggacttccacacggattctctgcagaaattgcacttcagctcggaccagatgtcacagtgattgactgtgcagctgactttcgtctgcaaaatgctgcagattgggagaagttctacggctcagagcaccagggaacatggccttatggcattccagaaataccaggacaccgcgaggctcttcgtggtgctaagcgtgtagcagtgccaggatgtttcccaaccggtgcaaccttggctcttcttcctgcggttcaagcgggacttatcgagccagatgtttccgtagtgtccatcaccggcgtatcaggtgcaggtaagaaagcatctgttgcactacttggctcggaaaccatgggttcactcaagacgtacaacacctccggaaagcaccgccacaccccggaaattgcccagaacctcggcgaagtcagcgacaagccagtcaaggtgagcttcaccccagtgcttgcaccgttacctcgcggaattctcaccactgcaaccgcacctttgaaagaaggcgttaccgcagagcaggctcgcgcagtatatgaagagttctatgcacaggaaaccttcgtgcatgttcttccagaaggtgcacagccacaaacccaagcagttcttggctccaacatgtgccacgtgcaggtagaaattgatgaggaagcaggcaaagtccttgttacctccgcaatcgataacctcaccaagggaactgccggcgccgctgttcagtgcatgaacttaagcgttggctttgatgaggcagcaggcctgccacaggtcggcgtcgcaccttaa

SEQ ID NO: 24 - DNA, 42 bp, synthetic construct
  source 1..42: mol_type = other DNA
gtgaattcgagctcggtacccgccccgaaaagccgttaaaag

SEQ ID NO: 25 - DNA, 42 bp, synthetic construct
  source 1..42: mol_type = other DNA
tgccaaaattcacgattattgcccacctacagctaaaactgc

SEQ ID NO: 26 - DNA, 42 bp, synthetic construct
  source 1..42: mol_type = other DNA
ttattggaggagatcaaaacaatgacaatcaaggttgcaatc

SEQ ID NO: 27 - DNA, 42 bp, synthetic construct
  source 1..42: mol_type = other DNA
ttaaggtgcgacgccgacctgggggatcctctagagtcgacc

SEQ ID NO: 28 - DNA, 21 bp, synthetic construct
  source 1..21: mol_type = other DNA
caataatcgtgaattttggca

SEQ ID NO: 29 - DNA, 21 bp, synthetic construct
  source 1..21: mol_type = other DNA
tgttttgatctcctccaataa

SEQ ID NO: 30 - protein, 500 aa, Corynebacterium glutamicum
MSDSPKNAPRITDEADVVLIGAGIMSSTLGAMLRQLEPSWTQIVFERLDGPAQESSSPWNNAGTGHSALCELNYTPEVKGKVEIAKAVGINEKFQVSRQFWSHLVEEGVLSDPKEFINPVPHVSFGQGADQVAYIKARYEALKDHPLFQGMTYADDEATFTEKLPLMAKGRDFSDPVAISWIDEGTDINYGAQTKQYLDAAEVEGTEIRYGHEVKSIKADGAKWIVTVKNVHTGDTKTIKANFVFVGAGGYALDLLRSAGIPQVKGFAGFPVSGLWLRCTNEELIEQHAAKVYGKASVGAPPMSVPHLDTRVIEGEKGLLFGPYGGWTPKFLKEGSYLDLFKSIRPDNIPSYLGVAAQEFDLTKYLVTEVLKDQDKRMDALREYMPEAQNGDWETIVAGQRVQVIKPAGFPKFGSLEFGTTLINNSEGTIAGLLGASPGASIAPSAMIELLERCFGDRMIEWGDKLKDMIPSYGKKLASEPALFEQQWARTQKTLKLEEA

SEQ ID NO: 31 - DNA, 1503 bp, Corynebacterium glutamicum
  source 1..1503: mol_type = genomic DNA
atgtcagattccccgaagaacgcaccgaggattaccgatgaggcagatgtagttctcattggtgccggtatcatgagctccacgctgggtgcaatgctgcgtcagctggagccaagctggactcagatcgtcttcgagcgtttggatggaccggcacaagagtcgtcctccccgtggaacaatgcaggaaccggccactctgctctatgcgagctgaactacaccccagaggttaagggcaaggttgaaattgccaaggctgtaggaatcaacgagaagttccaggtttcccgtcagttctggtctcacctcgttgaagagggagtgctgtctgatcctaaggaattcatcaaccctgttcctcacgtatctttcggccagggcgcagatcaggttgcatacatcaaggctcgctacgaagctttgaaggatcacccactcttccagggcatgacctacgctgacgatgaagctaccttcaccgagaagctgcctttgatggcaaagggccgtgacttctctgatccagtagcaatctcttggatcgatgaaggcaccgacatcaactacggtgctcagaccaagcagtacctggatgcagctgaagttgaaggcactgaaatccgctatggccacgaagtcaagagcatcaaggctgatggcgcaaagtggatcgtgaccgtcaagaacgtacacactggcgacaccaagaccatcaaggcaaacttcgtgttcgtcggcgcaggcggatacgcactggatctgcttcgcagcgcaggcatcccacaggtcaagggcttcgctggattcccagtatccggcctgtggcttcgttgcaccaacgaggaactgatcgagcagcacgcagccaaggtatatggcaaggcatctgttggcgctcctccaatgtctgttcctcaccttgacacccgcgttatcgagggtgaaaagggtctgctctttggaccttacggtggctggacccctaagttcttgaaggaaggctcctacctggacctgttcaagtccatccgcccagacaacattccttcctaccttggcgttgctgctcaggaatttgatctgaccaagtaccttgtcactgaagttctcaaggaccaggacaagcgtatggatgctcttcgcgagtacatgccagaggcacaaaacggcgattgggagaccatcgttgccggacagcgtgttcaggttattaagcctgcaggattccctaagttcggttccctggaattcggcaccaccttgatcaacaactccgaaggcaccatcgccggattgctcggtgcttcccctggagcatccatcgcaccttccgcaatgatcgagctgcttgagcgttgcttcggtgaccgcatgatcgagtggggcgacaagctgaaggacatgatcccttcctacggcaagaagcttgcttccgagccagcactgtttgagcagcagtgggcacgcacccagaagaccctgaagcttgaggaagcctaa

SEQ ID NO: 32 - protein, 500 aa, Corynebacterium glutamicum
MSDSPKNAPRITDEADVVLIGAGIMSSTLGAMLRQLEPSWTQIVFERLDGPAQESSSPWNNAGTGHSALCELNYTPEVKGKVEIAKAVGINEKFQVSRQFWSHLVEEGVLADPKEFINPVPHVSFGQGADQVAYIKARYEALKDHPLFQGMTYADDEATFTEKLPLMAKGRDFSDPVAISWIDEGTDINYGAQTKQYLDASEVEGTEIRYGHEVKSIKADGAKWIVTVKNVHTGDTKTIKANFVFVGAGGYALDLLRSAGIPQVKGFAGFPVSGLWLRCTNEELIEQHAAKVYGKASVGAPPMSVPHLDTRVIEGEKGLLFGPYGGWTPKFLKEGSYLDLFKSIRPDNIPSYLGVAAQEFDLTKYLVTEVLKDQDKRMDALREYMPEAQNGDWETIVAGQRVQVIKPAGFPKFGSLEFGTTLINNSEGTIAGLLGASPGASIAPSAMIELLERCFGDRMIEWGDKLKDMIPSYGKKLASEPALFEQQWARTQKTLKLEEA

SEQ ID NO: 33 - DNA, 1503 bp, Corynebacterium glutamicum
  source 1..1503: mol_type = genomic DNA
atgtcagattccccgaagaacgcaccgaggattaccgatgaggcagatgtagttctcattggtgccggtatcatgagctccacgctgggtgcaatgctgcgtcagctggagccaagctggactcagatcgtcttcgagcgtttggatggaccggcacaagagtcgtcctccccgtggaacaatgcaggaaccggccactctgctctatgcgagctgaactacaccccagaggttaagggcaaggttgaaattgccaaggctgtaggaatcaacgagaagttccaggtttcccgtcagttctggtctcacctcgttgaagagggcgtgctggctgatcctaaggaattcatcaaccctgttcctcacgtatctttcggccagggcgcagaccaggttgcatacatcaaggctcgctacgaagctttgaaggatcacccactcttccagggcatgacctacgctgacgatgaagctaccttcaccgagaagctgcctttgatggcaaagggccgtgacttctctgatccagtagcaatctcttggatcgatgaaggcaccgacatcaactacggtgctcagaccaagcagtacctggatgcatctgaagttgaaggcactgaaatccgctatggccacgaagtcaagagcatcaaggctgatggcgcaaagtggatcgtgaccgtcaagaacgtacacactggcgacaccaagaccatcaaggcaaacttcgtgttcgtcggcgcaggcgggtacgcactggatctgcttcgcagcgcaggcatcccacaggtcaagggcttcgctggattcccagtatccggcctgtggcttcgttgcaccaacgaggaactgatcgagcagcacgcagccaaggtatatggcaaggcatctgttggcgctcctccaatgtctgttcctcaccttgacacccgcgttatcgagggtgaaaagggtctgctctttggaccttacggtggctggacccctaagttcttgaaggaaggctcctacctggacctgttcaagtccatccgcccagacaacattccttcctaccttggcgttgctgctcaggaatttgatctgaccaagtaccttgtcactgaagttctcaaggaccaggacaagcgtatggatgctcttcgcgagtacatgccagaggcacaaaacggcgattgggagaccatcgttgccggacagcgtgttcaggttattaagcctgcaggattccctaagttcggttccctggaattcggcaccaccttgatcaacaactccgaaggcaccatcgccggattgctcggtgcttcccctggagcatccatcgcaccttccgcaatgatcgagctgcttgagcgttgcttcggtgaccgcatgatcgagtggggcgacaagctgaaggacatgatcccttcctacggcaagaagcttgcttccgagccagcactgtttgagcagcagtgggcacgcacccagaagaccctgaagcttgaggaagcctaa

SEQ ID NO: 34 - protein, 328 aa, Corynebacterium glutamicum
MNSPQNVSTKKVTVTGAAGQISYSLLWRIANGEVFGTDTPVELKLLEIPQALGGAEGVAMELLDSAFPLLRNITITADANEAFDGANAAFLVGAKPRGKGEERADLLANNGKIFGPQGKAINDNAADDIRVLVVGNPANTNALIASAAAPDVPASRFNAMMRLDHNRAISQLATKLGRGSAEFNNIVVWGNHSATQFPDITYATVGGEKVTDLVDHDWYVEEFIPRVANRGAEIIEVRGKSSAASAASSAIDHMRDWVQGTEAWSSAAIPSTGAYGIPEGIFVGLPTVSRNGEWEIVEGLEISDFQRARIDANAQELQAEREAVRDLL

SEQ ID NO: 35 - DNA, 987 bp, Corynebacterium glutamicum
  source 1..987: mol_type = genomic DNA
atgaattccccgcagaacgtctccaccaagaaggtcaccgtcaccggcgcagctggtcaaatctcttattcactgttgtggcgcatcgccaacggtgaagtattcggcaccgacacccctgtagaactgaaacttctggagatccctcaggctcttggcggggcagagggtgtggctatggaacttctggattctgccttccccctcctgcgaaacatcaccatcaccgcggatgccaatgaggcattcgacggcgctaatgcggcgtttttggtcggtgcgaagcctcgcggaaaaggcgaagagcgcgcagatttgctggctaacaacggcaagattttcggacctcaaggtaaagctatcaatgacaacgccgcagatgacattcgtgtcctagttgttggaaacccagcgaacaccaacgcgttgattgcttcagctgcggccccagatgttccagcatcccgcttcaacgcaatgatgcgccttgatcacaaccgtgcgatctcccagctggccaccaagcttggccgtggatctgcggaatttaacaacattgtggtctggggaaatcactccgcaacccagttcccagacatcacctacgcaaccgttggtggagaaaaggtcactgacctggttgatcacgattggtatgtggaggagttcattcctcgcgtggctaaccgtggcgctgaaatcattgaggtccgtggaaagtcttctgcagcttctgcagcatcctctgcgattgatcacatgcgcgattgggtacagggcaccgaggcgtggtcctctgcggcaattccttccaccggtgcatacggcattcctgagggcatttttgtcggtctgccaaccgtatcccgcaacggtgagtgggaaatcgttgaaggcctggagatttccgatttccagcgcgcccgcatcgacgcgaatgctcaggaattgcaggccgagcgcgaggcagtgcgcgacttgctctaa

SEQ ID NO: 36 - protein, 426 aa, Corynebacterium glutamicum
MSSVSLQDFDAERIGLFHEDIKRKFDELKSKNLKLDLTRGKPSSEQLDFADELLALPGKGDFKAADGTDVRNYGGLDGIVDIRQIWADLLGVPVEQVLAGDASSLNIMFDVISWSYIFGNNDSVQPWSKEETVKWICPVPGYDRHFSITERFGFEMISVPMNEDGPDMDAVEELVKNPQVKGMWVVPVFSNPTGFTVTEDVAKRLSAMETAAPDFRVVWDNAYAVHTLTDEFPEVIDIVGLGEAAGNPNRFWAFTSTSKITLAGAGVSFFLTSAENRKWYTGHAGIRGIGPNKVNQLAHARYFGDAEGVRAVMRKHAASLAPKFNKVLEILDSRLAEYGVAQWTVPAGGYFISLDVVPGTASRVAELAKEAGIALTGAGSSYPLRQDPENKNLRLAPSLPPVEELEVAMDGVATCVLLAAAEHYAN

SEQ ID NO: 37 - DNA, 1281 bp, Corynebacterium glutamicum
  source 1..1281: mol_type = genomic DNA
atgagttcagtttcgctgcaggattttgatgcagagcgaattggtttgttccacgaggacattaagcgcaagtttgatgagctcaagtcaaaaaatctgaagctggatcttactcgcggtaagccttcgtcggagcagttggatttcgctgatgagttgttggcgttgcctggtaagggtgatttcaaggctgcggatggtactgatgtccgtaactatggcgggctggatggcatcgttgatattcgccagatttgggcggatttgctgggtgttcctgtggagcaggtcttggcgggggatgcttcgagcttgaacatcatgtttgatgtgatcagctggtcgtacattttcggtaacaatgattcggttcagccttggtcgaaggaagaaaccgttaagtggatttgccctgttccgggctatgatcgccatttctccatcacggagcgtttcggctttgagatgatttctgtgccaatgaatgaagacggccctgatatggatgctgttgaggaattggtgaagaatccgcaggttaagggcatgtgggttgttccggtgttttctaacccgactggtttcacggtgacagaagacgtcgcaaagcgtctaagcgcaatggaaaccgcagctccggacttccgcgttgtgtgggataatgcctacgccgttcatacgctgaccgatgaattccctgaggttatcgatatcgtcgggcttggtgaggccgctggcaacccgaaccgtttctgggcgttcacttctacttcgaagatcactctcgcgggtgcgggcgtgtcgttcttcctcacctctgcggagaaccgcaagtggtacaccggccatgcgggtatccgtggcattggccctaacaaggtcaatcagttggctcatgcgcgttactttggcgatgctgagggagtgcgcgcggtgatgcgtaagcatgctgcgtcgttggctccgaagttcaacaaggttctggagattctggattctcgccttgctgagtacggtgtcgcgcagtggactgtccctgcgggcggttacttcatttcccttgatgtggttcctggtacggcgtctcgcgtggctgagttggctaaggaagccggcatcgcgttgacgggtgcgggttcttcttacccgctgcgtcaggatccggagaacaaaaatctccgtttggcaccgtcgctgcctccagttgaggaacttgaggttgccatggatggcgtggctacctgtgtgctgttggcagcagcggagcattacgctaactaa

SEQ ID NO: 38 - protein, 447 aa, Corynebacterium glutamicum
MTVDEQVSNYYDMLLKRNAGEPEFHQAVAEVLESLKIVLEKDPHYADYGLIQRLCEPERQLIFRVPWVDDQGQVHVNRGFRVQFNSALGPYKGGLRFHPSVNLGIVKFLGFEQIFKNSLTGLPIGGGKGGSDFDPKGKSDLEIMRFCQSFMTELHRHIGEYRDVPAGDIGVGGREIGYLFGHYRRMANQHESGVLTGKGLTWGGSLVRTEATGYGCVYFVSEMIKAKGESISGQKIIVSGSGNVATYAIEKAQELGATVIGFSDSSGWVHTPNGVDVAKLREIKEVRRARVSVYADEVEGATYHTDGSIWDLKCDIALPCATQNELNGENAKTLADNGCRFVAEGANMPSTPEAVEVFRERDIRFGPGKAANAGGVATSALEMQQNASRDSWSFEYTDERLQVIMKNIFKTCAETAAEYGHENDYVVGANIAGFKKVADAMLAQGVI

SEQ ID NO: 39 - DNA, 1344 bp, Corynebacterium glutamicum
  source 1..1344: mol_type = genomic DNA
atgacagttgatgagcaggtctctaactattacgacatgcttctgaagcgcaatgctggcgagcctgaatttcaccaggcagtggcagaggttttggaatctttgaagatcgtcctggaaaaggaccctcattacgctgattacggtctcatccagcgcctgtgcgagcctgagcgtcagctcatcttccgtgtgccttgggttgatgaccagggccaggtccacgtcaaccgtggtttccgcgtgcagttcaactctgcacttggaccatacaagggcggcctgcgcttccacccatctgtaaacctgggcattgtgaagttcctgggctttgagcagatctttaaaaactccctaaccggcctgccaatcggtggtggcaagggtggatccgacttcgaccctaagggcaagtccgatctggaaatcatgcgtttctgccagtccttcatgaccgagctacaccgccacatcggtgagtaccgcgacgttcctgcaggtgacatcggagttggtggccgcgagatcggttacctgtttggccactaccgtcgcatggctaaccagcacgagtccggcgttttgaccggtaagggcctgacctggggtggatccctggtccgcaccgaggcaactggctacggctgcgtttacttcgtgagtgaaatgatcaaggctaagggcgagagcatcagcggccagaagatcatcgtttccggttccggcaacgtagcaacctacgcgattgaaaaggctcaggaactcggcgcaaccgttattggtttctccgattccagcggttgggttcatacccctaacggcgttgacgtggctaagctccgcgaaatcaaggaagttcgtcgcgcacgcgtatccgtgtacgccgacgaagttgaaggcgcaacctaccacaccgacggttccatctgggatctcaagtgcgatatcgctcttccttgtgcaactcagaacgagctcaacggcgagaacgctaagactcttgcagacaacggctgccgtttcgttgctgaaggcgcgaacatgccttccacccctgaggctgttgaggtcttccgtgagcgcgacatccgcttcggaccaggcaaggcagctaacgctggtggcgttgcaacctccgctctggagatgcagcagaacgcttcgcgcgattcctggagcttcgagtacaccgacgagcgcctccaggtgatcatgaagaacatcttcaagacctgtgcagagaccgcagcagagtatggacacgagaacgattacgttgtcggcgctaacattgctggcttcaagaaggtagctgacgcgatgctggcacagggcgtcatctaa

SEQ ID NO: 40 - protein, 469 aa, Corynebacterium glutamicum; identical to SEQ ID NO: 1

SEQ ID NO: 41 - DNA, 1410 bp, Corynebacterium glutamicum
  source 1..1410: mol_type = genomic DNA
atgaccgagcaggaattccgtattgagcacgacaccatgggtgaagtgaaggttccagcaaaggctctgtggcaggcacagacccagcgcgctgttgagaacttccctatctctggtcgtggtctggaatccgcacagatccgcgcaatgggtctgctgaaggcagcttgtgcgcaggtaaacaaggactccggtgcgctggatgcagagaaggcagatgccatcattgcagctggtaaggagatcgcgtccggtaagcatgacgctgagttcccaattgatgtgttccagactggttccggtacttcctccaacatgaacaccaatgaggttatcgcttccatcgcgaaggctaacggcgttgaggttcacccaaatgaccacgtcaacatgggtcagtcctccaatgacaccttccctactgcaactcacgttgctgcaaccgaagctgctgtcaatgacctcatcccaggcctgaaggttctgcacgagtctttggcgaagaaggctaacgagtggtctgaggttgttaagtccggccgcacccacctgatggacgctgttccagtaaccctgggccaggagttcggtggctacgctcgccagatccagctcggcatcgagcgcgttgaggctactcttcctcgccttggtgagctggctattggtggcaccgctgctggtaccggtatcaacacctccgctgatttcggcggcaaggttgttgctgaactgatcaacttgaccgacgtcaaggagctcaaggaagctgagaaccacttcgaggctcaggctgcacgcgacgctcttgttgagttctccggcgcaatgcgcgttatcgctgtctccttgtacaagatcgctaacgatatccgcctcatgggctccggcccactgaccggtcttggcgagatccgtctcccagacctgcagccaggttcctccatcatgccaggcaaggtcaacccagttctctgtgagaccgctacccaggtttccgctcaggttatcggcaatgacgcagctgttgcgttctccggcacccagggccagttcgagctcaacgtgttcatcccagtgatggctcgcaacgtgcttgagtccgctcgcctgctggctaacacttcccgcgtgttcgcaacccgtctcgttgatggcattgagccaaacgaggcacacatgaaggagctcgctgagtcttcaccttccatcgttaccccactgaactctgcaatcggctacgaagctgctgcaaaggtggctaagactgctttggctgagggcaagaccatccgccagactgtcatcgatttgggcttggttgatggcgagaagctcaccgaggaagagctggacaagcgcctcgacgttcttgctatggctcacaccgagcgcgagaacaagttctaa

SEQ ID NO: 42 - DNA, 42 bp, synthetic construct
  source 1..42: mol_type = other DNA
gtgaattcgagctcggtacccatactactcatgtttgcgaat

SEQ ID NO: 43 - DNA, 42 bp, synthetic construct
  source 1..42: mol_type = other DNA
tcctgatatcgggcaccatttggcaaagaatacgcaaagcac

SEQ ID NO: 44 - DNA, 41 bp, synthetic construct
  source 1..41: mol_type = other DNA
tgctttgcgtattctttgccaaatggtgcccgatatcagga

SEQ ID NO: 45 - DNA, 42 bp, synthetic construct
  source 1..42: mol_type = other DNA
aacaaagcagccatgcgttgcagccgttacttaaaccaagtc

SEQ ID NO: 46 - DNA, 43 bp, synthetic construct
  source 1..43: mol_type = other DNA
cgacttggtttaagtaacggctgcaacgcatggctgctttgtt

SEQ ID NO: 47 - DNA, 42 bp, synthetic construct
  source 1..42: mol_type = other DNA
gcgaatgagaccagttgactgttagttagcgtaatgctccgc

SEQ ID NO: 48 - DNA, 42 bp, synthetic construct
  source 1..42: mol_type = other DNA
gcggagcattacgctaactaacagtcaactggtctcattcgc

SEQ ID NO: 49 - DNA, 42 bp, synthetic construct
  source 1..42: mol_type = other DNA
ggttaatatccaatatggaagttagatgacgccctgtgccag

SEQ ID NO: 50 - DNA, 42 bp, synthetic construct
  source 1..42: mol_type = other DNA
ctggcacagggcgtcatctaacttccatattggatattaacc

SEQ ID NO: 51 - DNA, 42 bp, synthetic construct
  source 1..42: mol_type = other DNA
attcgcaaacatgagtagtatttagaacttgttctcgcgctc

SEQ ID NO: 52 - DNA, 41 bp, synthetic construct
  source 1..41: mol_type = other DNA
cgcgagaacaagttctaaatactactcatgtttgcgaattg

SEQ ID NO: 53 - DNA, 42 bp, synthetic construct
  source 1..42: mol_type = other DNA
ggtcgactctagaggatccccttaggcttcctcaagcttcag

SEQ ID NO: 54 - DNA, 15 bp, synthetic construct
  source 1..15: mol_type = other DNA
ctcttcaccagcatt

SEQ ID NO: 55 - DNA, 20 bp, synthetic construct
  source 1..20: mol_type = other DNA
ttgtcacaacatctgtttca

SEQ ID NO: 56 - protein, 454 aa, Corynebacterium glutamicum
MFTASIPTYELGSFSKGSYVEIKGTYFYPDTLNTLFRNSGAKDNEEFFVDVTLVPEPDNPHSTRGHAISVRWNDLVIGHIASDMTEKFQQVRRVAASGYDARVSARIWTNTNYKNERDFWVSVKLPDPDFLVPLNDPPHDGFTLLPYGTAIQVTKESDHMDVLSEFVPPSGQGQILVSLHIINAGVRKEWDGIEVRLDNQRIGELTKASSEKFAPVVRHFDDLGLSTLCRALIKGSSLAAEVTLYGARAHELSEEDLEPKSSSPLPRLVEYQSNPFNYQVPNRWPGEQNQRAPKSQKSSSSPFAAYRGPSQPSKSLTPFVAQTPAPQPSDRFIDWDSLLQPDGTPRATPFQRGVTRGLIGKHFSNQKSPRIDFATVGQCDAILRTFGEPTDKLYKDGRTSWPLWWALMAIVTLLVMLLNFIPGIGPIFPLIGLIVLGHHFWTRRKLNPPFGRSK

SEQ ID NO: 57 - DNA, 1365 bp, Corynebacterium glutamicum
  source 1..1365: mol_type = genomic DNA
atgtttaccgcatccattcctacttatgaattagggtctttcagcaagggctcctacgttgagatcaaaggaacttacttctaccctgacacgctaaatactttatttagaaattctggggcaaaagacaacgaagagttctttgtagacgtaactcttgttccagaaccagataatccgcatagcactcgaggccatgccatttcagtccgctggaatgatctcgtaataggacatattgcctcggatatgactgaaaaattccaacaagtgcgacgagttgcagctagtggctacgatgctcgagtctctgctcggatttggacgaatacaaactataagaatgaacgagatttttgggtatctgttaagctccccgatccagatttccttgttcctcttaatgatcctccccatgacgggtttaccctcctcccttatggaacagcaatccaagtcaccaaggaatctgatcacatggacgtgctctcagaattcgtgcctccatctggacaaggtcagattctcgtatcgctacacatcattaacgcaggcgtgagaaaagaatgggatggcattgaagttcggctcgataatcaacggatcggagagcttacaaaggccagttcagaaaaattcgcacccgtagtgcgacatttcgatgacctaggacttagtacactatgtcgtgcgctcatcaaggggtcatcactagctgctgaagtaactctatatggagctcgtgcacatgagctttccgaagaagacttagaacctaaaagctcttccccattgcccaggttggttgaataccagtcaaatccgtttaattatcaagtccccaacaggtggcccggcgagcagaatcaacgtgctcctaagtcgcaaaagtcttcttcatcacctttcgcagcgtatcgcgggccatcgcaacctagtaaatcactcacaccgtttgtagcgcagacacctgcgcctcagcctagtgatcgatttattgattgggattcattgcttcaaccggacggaactccaagagctacgccattccaaagaggagtaacccgcgggttaattggcaagcatttttcgaatcaaaaatctccaagaattgactttgcaacggtggggcaatgtgatgcaattctccgaactttcggagagccgaccgacaagctttataaagacggcaggacttcttggcctttgtggtgggcgctcatggcgatagtcacccttctcgtcatgttgctgaactttattccaggaattggtccgatcttcccacttatcggattgatcgtacttggtcatcacttttggactcgccgaaaacttaacccaccattcggtagatcaaaatag

SEQ ID NO: 58 - DNA, 44 bp, synthetic construct
  source 1..44: mol_type = other DNA
agtgaattcgagctcggtacccgcgacatttcgatgacctagga

SEQ ID NO: 59 - DNA, 36 bp, synthetic construct
  source 1..36: mol_type = other DNA
agagtggcagcagtcccgggagggaaattagtcaga

SEQ ID NO: 60 - DNA, 42 bp, synthetic construct
  source 1..42: mol_type = other DNA
tgactaatttccctcccgggactgctgccactctcactgctt

SEQ ID NO: 61 - DNA, 42 bp, synthetic construct
  source 1..42: mol_type = other DNA
ggtcgactctagaggatcccctacagtgcttcagtatcggta

SEQ ID NO: 62 - DNA, 40 bp, synthetic construct
  source 1..40: mol_type = other DNA
ttattggaggagatcaaaacaatgaccgagcaggaattcc

SEQ ID NO: 63 - DNA, 37 bp, synthetic construct
  source 1..37: mol_type = other DNA
agagtggcagcagtcccttagaacttgttctcgcgct

SEQ ID NO: 64 - DNA, 37 bp, synthetic construct
  source 1..37: mol_type = other DNA
tgactaatttccctcccggcgcttcatgtcaacaatc

SEQ ID NO: 65 - DNA, 39 bp, synthetic construct
  source 1..39: mol_type = other DNA
ggaattcctgctcggtcattgttttgatctcctccaata

SEQ ID NO: 66 - protein, 377 aa, Corynebacterium glutamicum
MPTLAPSGQLEIQAIGDVSTEAGAIITNAEIAYHRWGEYRVDKEGRSNVVLIEHALTGDSNAADWWADLLGPGKAINTDIYCVICTNVIGGCNGSTGPGSMHPDGNFWGNRFPATSIRDQVNAEKQFLDALGITTVAAVLGGSMGGARTLEWAAMYPETVGAAAVLAVSARASAWQIGIQSAQIKAIENDHHWHEGNYYESGCNPATGLGAARRIAHLTYRGELEIDERFGTKAQKNENPLGPYRKPDQRFAVESYLDYQADKLVQRFDAGSYVLLTDALNRHDIGRDRGGLNKALESIKVPVLVAGVDTDILYPYHQQEHLSRNLGNLLAMAKIVSPVGHDAFLTESRQMDRIVRNFFSLISPDEDNPSTYIEFYI

SEQ ID NO: 67 - DNA, 1134 bp, Corynebacterium glutamicum
  source 1..1134: mol_type = genomic DNA
atgcccaccctcgcgccttcaggtcaacttgaaatccaagcgatcggtgatgtctccaccgaagccggagcaatcattacaaacgctgaaatcgcctatcaccgctggggtgaataccgcgtagataaagaaggacgcagcaatgtcgttctcatcgaacacgccctcactggagattccaacgcagccgattggtgggctgacttgctcggtcccggcaaagccatcaacactgatatttactgcgtgatctgtaccaacgtcatcggtggttgcaacggttccaccggacctggctccatgcatccagatggaaatttctggggtaatcgcttccccgccacgtccattcgtgatcaggtaaacgccgaaaaacaattcctcgacgcactcggcatcaccacggtcgccgcagtacttggtggttccatgggtggtgcccgcaccctagagtgggccgcaatgtacccagaaactgttggcgcagctgctgttcttgcagtttctgcacgcgccagcgcctggcaaatcggcattcaatccgcccaaattaaggcgattgaaaacgaccaccactggcacgaaggcaactactacgaatccggctgcaacccagccaccggactcggcgccgcccgacgcatcgcccacctcacctaccgtggcgaactagaaatcgacgaacgcttcggcaccaaagcccaaaagaacgaaaacccactcggtccctaccgcaagcccgaccagcgcttcgccgtggaatcctacttggactaccaagcagacaagctagtacagcgtttcgacgccggctcctacgtcttgctcaccgacgccctcaaccgccacgacattggtcgcgaccgcggaggcctcaacaaggcactcgaatccatcaaagttccagtccttgtcgcaggcgtagataccgatattttgtacccctaccaccagcaagaacacctctccagaaacctgggaaatctactggcaatggcaaaaatcgtatcccctgtcggccacgatgctttcctcaccgaaagccgccaaatggatcgcatcgtgaggaacttcttcagcctcatctccccagacgaagacaacccttcgacctacatcgagttctacatctaa

SEQ ID NO: 68 - DNA, 28 bp, synthetic construct
  source 1..28: mol_type = other DNA
ggatcccctcgttgttcacccagcaacc

SEQ ID NO: 69 - DNA, 30 bp, synthetic construct
  source 1..30: mol_type = other DNA
ggatcccaaagtcacaactacttatgttag

SEQ ID NO: 70 - protein, 436 aa, Corynebacterium glutamicum
MKSTGNIIADTICRTAELGLTITGASDAGDYTLIEADALDYTSTCPECSQPGVFRHHTHRMLIDLPIVGFPTKLFIRLPRYRCTNPTCKQKYFQAELSCADHGKKVTHRVTRWILQRLAIDRMSVHATAKALGLGWDLTCQLALDMCRELVYNDPHHLDGVYVIGVDEHKWSHNRAKHGDGFVTVIVDMTGHRYDSRCPARLLDVVPGRSADALRSWLGSRGEQFRNQIRIVSMDGFQGYATASKELIPSARRVMDPFHVVRLAGDKLTACRQRLQREKYQRRGLSQDPLYKNRKTLLTTHKWLSPRQQESLEQLWAYDKDYGALKLAWLAYQAIIDCYQMGNKREAKKKMRTIIDQLRVLKGPNKELAQLGRSLFKRLGDVLAYFDVGVSNGPVEAINGRLEHLRGIALGFRNLNHYILRCLIHSGQLVHKINAL

SEQ ID NO: 71 - DNA, 1311 bp, Corynebacterium glutamicum
  source 1..1311: mol_type = genomic DNA
atgaagtctaccggcaacatcatcgctgacaccatctgccgcactgcggaactaggactcaccatcaccggcgcttccgatgcaggtgattacaccctgatcgaagcagacgcactcgactacacctccacctgcccagaatgctcccaacctggggtgtttcgtcatcacacccaccggatgctcattgatttacccatcgtcgggtttcccaccaaactgtttatccgtctacctcgctaccgctgcaccaaccccacatgtaagcaaaagtatttccaagcagaactaagctgcgctgaccacggtaaaaaggtcacccaccgggtcacccgctggattttacaacgccttgctattgaccggatgagtgttcacgcaaccgcgaaagcacttgggctagggtgggatttaacctgccaactagccctcgatatgtgccgtgagctggtctataacgatcctcaccatcttgatggagtgtatgtcattggggtggatgagcataagtggtcacataatagggctaagcatggtgatgggtttgtcaccgtgattgtcgatatgaccgggcatcggtatgactcacggtgtcctgcccggttattagatgtcgtcccaggtcgtagtgctgatgctttacggtcctggcttggctcccgcggtgaacagttccgcaatcagatacggatcgtgtccatggatggattccaaggctacgccacagcaagtaaagaactcattccttctgctcgtcgcgtgatggatccattccatgttgtgcggcttgctggtgacaagctcaccgcctgccggcaacgcctccagcgggagaaataccagcgtcgtggtttaagccaggatccgttgtataaaaaccggaagaccttgttgaccacgcacaagtggttgagtcctcgtcagcaagaaagcttggagcagttgtgggcgtatgacaaagactacggggcgttaaagcttgcgtggcttgcgtatcaggcgattattgattgttatcagatgggtaataagcgtgaagcgaagaagaaaatgcggaccattattgatcagcttcgggtgttgaaggggccgaataaggaactcgcgcagttgggtcgtagtttgtttaaacgacttggtgatgtgttggcgtatttcgatgttggtgtctccaacggtccggtcgaagcgatcaacggacggttggagcatttgcgtgggattgctctaggtttccgtaatttgaaccactacattctgcggtgccttatccattcagggcagttggtccataagatcaatgcactctaa

SEQ ID NO: 72 - protein, 87 aa, Corynebacterium glutamicum
MKTFDSLYEELLNRAQTRPEGSGTVAALDKGIHHLGKKVIEEAGEVWIAAEYETDEELAGEISQLIYWTQVIMVARGLKPEDIYKNL

SEQ ID NO: 73 - DNA, 264 bp, synthetic construct
  source 1..264: mol_type = other DNA
atgaagacatttgactcgctgtacgaagaacttcttaaccgtgctcagacccgccctgaagggtctggaaccgtggccgccttggataaaggcatccatcatctaggtaagaaggtcatcgaagaagccggagaggtctggattgcagccgagtatgagaccgatgaagagctagccggagaaatctcccagctcatttattggacccaggtcatcatggttgctcgcggcctgaagccagaagatatctacaagaacctgtag

SEQ ID NO: 74 - protein, 281 aa, synthetic construct
MLKIAVPNKGSLSERAMEILAEAGYAGRGDSKSLNVFDEANNVEFFFLRPKDIAIYVAGGQLDLGITGRDLARDSQADVHEVLSLGFGSSTFRYAAPADEEWSIEKLDGKRIATSYPNLVRDDLAARGLSAEVLRLDGAVEVSIKLGVADAIADVVSTGRTLRQQGLAPFGEVLCTSEAVIVGRKDEKVTPEQQILLRRIQGILHAQNFLMLDYNVDRDNLDAATAVTPGLSHPQVSPLARDNWVAVRAMVPRRSANAIMDKLAGLGAEAILASEIRIARI

SEQ ID NO: 75 - DNA, 846 bp, synthetic construct
  source 1..846: mol_type = other DNA
atgttgaaaatcgctgtcccaaacaaaggctcgctgtccgagcgcgccatggaaatcctcgccgaagcaggctacgcaggccgtggagattccaaatccctcaacgtttttgatgaagcaaacaacgttgaattcttcttccttcgccctaaagatatcgccatctacgttgctggtggccagctcgatttgggtatcaccggccgcgaccttgctcgcgattcccaggctgatgtccacgaagttctttccctcggcttcggttcctccactttccgttacgcagcaccagctgatgaagagtggagcatcgaaaagctcgacggcaagcgcatcgctacctcttaccccaaccttgttcgcgatgacctcgcagcacgtgggctttccgctgaggtgctccgcctcgacggtgcagtagaggtatccatcaagcttggtgtcgcagatgccatcgccgatgttgtatccaccggccgcacgctgcgtcagcaaggtcttgcacctttcggcgaggttctgtgcacctctgaggctgtcattgttggccgcaaggatgaaaaggtcaccccagagcagcagatcctgcttcgccgcatccagggaattttgcacgcgcagaacttcctcatgctggattacaacgtcgaccgcgacaacctggacgctgccactgcagtaaccccaggcttatcccacccacaggtatccccactggcacgcgacaactgggttgctgtacgcgccatggtgccacgcaggtcagctaacgccatcatggataagcttgctggactcggcgctgaagccatcctggcttctgaaatccgcatcgcccgcatctag

SEQ ID NO: 76 - protein, 260 aa, Corynebacterium glutamicum
MSKYADDLALALELAELADSITLDRFEASDLEVSSKPDMTPVSDADLATEEALREKIATARPADSILGEEFGGDVEFSGRQWIIDPIDGTKNYVRGVPVWATLIALLDNGKPVAGVISAPALARRWWASEGAGAWRTFNGSSPRKLSVSQVSKLDDASLSFSSLSGWAERDLRDQFVSLTDTTWRLRGYGDFFSYCLVAEGAVDIAAEPEVSLWDLAPLSILVTEAGGKFTSLAGVDGPHGGDAVATNGILHDETLDRLK

SEQ ID NO: 77 - DNA, 783 bp, Corynebacterium glutamicum
  source 1..783: mol_type = genomic DNA
atgagcaaatatgcagacgatttagccttagccctcgaacttgccgaacttgccgattccatcaccctcgaccgcttcgaagcctctgacctggaagtatcctccaagccagacatgactcccgtcagcgatgccgacctggcgaccgaagaagcactccgtgagaaaatcgccaccgcccgccccgccgactccatcctcggtgaagaattcggtggcgacgtagaattcagcggccgccagtggatcatcgaccccatcgacggcaccaaaaactacgtccgcggcgtccccgtatgggcaaccctgatcgcgctgctcgacaacggcaaacccgtcgcaggtgtcatctccgcacccgcactggctaggcgttggtgggcatccgaaggggccggcgcatggcgcaccttcaacggcagctccccacgcaaactgtccgtgtcccaggtgtccaagcttgacgacgcctccctctccttctcctccctctccggctgggccgaacgagatttgcgcgatcagttcgtctccctaactgataccacctggcgactccgcggctacggcgacttcttctcctactgcctcgtcgccgaaggtgccgtcgatatcgccgctgaaccagaagtcagcctctgggatcttgctcccctgtccatcctggtcaccgaagccggaggaaagttcacctcactggctggcgtcgatggaccacacggtggcgatgcagtagccaccaacggcatcctgcacgatgagacgctggatcgtttaaaatag

SEQ ID NO: 78 - protein, 442 aa, Corynebacterium glutamicum
MLNVTDLRGQTPSKSDIRRALPRGGTDVWSVLPIVQPVVEDVQNRGAEAALDYGEKFDHIRPASVRVPAEVIAAAENTLDPLVRESIEESIRRVRKVHAEQKPSEHTTELSPGGTVTERFMPIDRVGLYVPGGNAVYPSSVIMNTVPAQEAGVNSLVVASPPQAEHGGWPHPTILAACSILGVDEVWAVGGGQAVALLAYGDDAAGLEPVDMITGPGNIFVTAAKRLVRGVVGTDSEAGPTEIAVLADASANAVNVAYDLISQAEHDVMAASVLITDSEQLAKDVNREIEARYSITRNAERVAEALRGAQSGIVLVDDISVGIQVADQYAAEHLEIHTENARAVAEQITNAGAIFVGDFSPVPLGDYSAGSNHVLPTSGSARFSAGLSTHTFLRPVNLIEYDEAALKDVSQVVINFANAEDLPAHGEAIRARFENLPTTDEA

SEQ ID NO: 79 - DNA, 1329 bp, Corynebacterium glutamicum
  source 1..1329: mol_type = genomic DNA
atgttgaatgtcactgacctgcgaggtcaaacaccatccaagagcgacatccgacgtgctttgccacgtggtggcactgacgtgtggtctgtgcttcccatagtgcagcctgttgtagaagatgtccaaaaccgcggcgctgaagctgctttggattacggcgagaagttcgaccatattcgccccgcctcggtgcgggtgccagctgaggttattgctgcagcagaaaacaccttagatccgttggtgcgtgaatcgattgaagagtcgattcgtcgcgtccgcaaggttcacgctgagcaaaagccatccgagcacaccactgaactttcaccaggtggcaccgtcactgagcgtttcatgccgattgatcgcgtgggactgtacgttccaggcggcaatgcggtgtacccatcaagcgtgattatgaatactgtcccagctcaagaggctggtgtgaactcccttgtggttgcgtcgcctcctcaggctgagcacggtggctggcctcaccccaccattttggcggcgtgttccatcttgggtgttgatgaggtgtgggctgtcggcggcggtcaggccgtggcgttgctggcttatggtgatgacgctgcaggtctcgagcctgtggatatgatcactggacctggcaatatctttgtcaccgctgcgaagcgcctggtcaggggagtggtaggtactgattctgaggctggccctacagaaatcgctgtgcttgctgatgcctctgccaacgccgtcaacgttgcctacgatctgatcagccaagcagaacacgatgtcatggctgcgtccgtgctcatcactgactccgagcagcttgccaaggacgtaaacagggaaatcgaggcgcgttactcaatcacgcgcaacgccgagcgcgtcgcagaagctttgcgcggggcccagagtggcatcgtgcttgtcgacgacatttccgtgggtatccaagtagccgatcaatacgcagcggaacacctggaaatccacactgagaacgcgcgcgccgtagcagagcagatcaccaacgcgggtgcgatcttcgtgggcgatttctcaccagtaccactgggtgattactccgcaggatccaaccacgtgctgccaacctctggatccgctcgtttctccgcaggtctatccacgcacacgttccttcgcccagtcaacctcattgaatacgatgaggctgctctgaaggacgtctcgcaggttgtcatcaactttgccaacgccgaagatcttccagcgcacggcgaagcaatccgtgcacgctttgaaaacctccccaccaccgacgaggcctaa

SEQ ID NO: 80 - protein, 246 aa, Corynebacterium glutamicum
MTFTILPAVDVVNGQAVRLDQGEAGTEKSYGTPLESALKWQEQGAKWLHFVDLDAAFNRGSNHEMMAEIVGKLDVDVELTGGIRDDESLERALATGARRVNIGTAALEKPEWIASAIQRYGEKIAVDIAVRLEDGEWRTRGNGWVSDGGDLWEVLERLDSQGCARFVVTDVSKDGTLSGPNVELLREVAAATDAPIVASGGISVLEDVLELAKYQDEGIDSVIIGKALYEHKFTLEEALAAVEKLG

SEQ ID NO: 81 - DNA, 741 bp, Corynebacterium glutamicum
  source 1..741: mol_type = genomic DNA
atgaccttcactattcttcctgcagtcgatgtagttaacggacaagcagttcgcctagatcagggcgaggccggcactgaaaagtcttatggcacccctttggaatccgcactgaagtggcaggagcagggtgcaaagtggttgcactttgtggacctggacgcagcgttcaaccgtggttccaaccatgagatgatggcggaaattgtcggcaagctcgatgttgatgtggagctcactggcggtatccgtgatgatgagtctctggagcgcgcgctggcaaccggtgcacgtcgtgtaaacattggtaccgctgctctggagaagccagagtggattgcttctgcgattcaacgctatggcgagaagattgctgtcgatatcgctgtgcgtttggaagatggtgaatggcgcacccgtggaaacggttgggtctccgatggtggcgatctgtgggaagttctcgagcgtttggattcccaaggttgtgcacgtttcgtggttaccgatgtgtccaaggacggcaccttgagtggtccaaatgttgagctgctgcgtgaggttgctgcagctacagacgcacctatcgtggcatctggtggaatttctgttttggaagatgttttggaactagccaagtaccaggatgagggcattgattccgtcatcattggcaaggcactttatgagcacaagttcaccctcgaagaggctttggctgcagtagaaaagctcggttaa

SEQ ID NO: 82 - protein, 202 aa, Corynebacterium glutamicum
MTVAPRIGTATRTTSESDITVEINLDGTGKVDIDTGLPFFDHMLTAFGVHGSFDLKVHAKGDIEIDAHHTVEDTAIVLGQALLDAIGDKKGIRRFASCQLPMDEALVESVVDISGRPYFVISGEPDHMITSVIGGHYATVINEHFFETLALNSRITLHVICHYGRDPHHITEAEYKAVARALRGAVEMDPRQTGIPSTKGAL

SEQ ID NO: 83 - DNA, 609 bp, Corynebacterium glutamicum
  source 1..609: mol_type = genomic DNA
atgactgtcgcaccaagaattggtaccgcaacccgcaccaccagcgaatccgacatcaccgtcgagatcaacctggacggcaccggcaaagtagatatcgataccggcctgccatttttcgaccacatgctcactgcattcggcgtgcacggcagttttgatctgaaagtccatgccaagggcgacatcgagatcgacgcacaccacaccgtggaagataccgccatcgtgctcggccaagcactccttgacgctattggcgacaagaaaggcatccgccgtttcgcatcctgccagctgcccatggatgaggcattagtggagtccgtggtggatatctccggtcgcccatacttcgtgatctccggcgaaccagaccacatgatcacctccgtgatcggtggacactacgcaaccgtgatcaacgagcacttctttgaaaccctcgcgctcaactcccgaatcaccctccacgtgatctgccactacggccgcgaccctcaccacatcaccgaagcagagtacaaggctgttgcccgtgcgctgcgcggtgccgtagagatggatcctcgtcaaacaggaatcccatccactaagggagcgctctag

SEQ ID NO: 84 - protein, 211 aa, Corynebacterium glutamicum
MTKTVALLDYGSGNLRSAQRALERAGAEVIVSSDPEVCTNADGLLVPGVGAFDACMKGLKNVFGHRIIGQRLAGGRPVMGICVGMQILFDEGDEHGIKSAGCGEWPGKVERLQAEILPHMGWNTLEMPTNSPMFEGISPDERFYFVHSYGVRKWTLETDDLTTPPEVVWAKHENDRFVAAVENGTLWATQFHPEKSGDAGAQLLRNWINYI

SEQ ID NO: 85 - DNA, 636 bp, Corynebacterium glutamicum
  source 1..636: mol_type = genomic DNA
atgaccaaaactgtcgcccttctcgactacggatctggaaaccttcgttctgctcaacgcgcactagagcgtgccggtgcagaagttatcgtgagctccgatccagaagtttgcaccaacgctgatggcctcctagttcctggagtgggcgcatttgatgcctgcatgaagggtttgaaaaacgtcttcggacatcgcattatcggacagcgtcttgctggtggacgtccagtgatgggtatttgtgtgggcatgcagatcctgttcgatgaaggcgatgagcacggcattaagtcagctggttgcggcgagtggcctggcaaagtggaacgcctccaagcggagatcctgcctcacatggggtggaacacacttgaaatgcctaccaactcaccaatgtttgagggaatttcacctgatgagcgtttctacttcgtgcactcctatggtgtgcgcaagtggacgttggaaaccgacgatctgaccacgcctccagaggttgtgtgggcgaagcacgaaaatgatcgttttgtggcagctgtggaaaacggcacgctgtgggctactcaattccacccagaaaaatcaggtgacgcaggcgcacagctactgcgaaactggatcaactacatctaa

SEQ ID NO: 86 - DNA, 30 bp, synthetic construct
  source 1..30: mol_type = other DNA
gaggagatcaaaacagtgaagacatttgac

SEQ ID NO: 87 - DNA, 30 bp, synthetic construct
  source 1..30: mol_type = other DNA
acaccaagcttgatggatacctctactgca

SEQ ID NO: 88 - DNA, 29 bp, synthetic construct
  source 1..29: mol_type = other DNA
cagtagaggtatccatcaagcttggtgtc

SEQ ID NO: 89 - DNA, 28 bp, synthetic construct
  source 1..28: mol_type = other DNA
actctagaggatccccctagatgcgggc

SEQ ID NO: 90 - DNA, 34 bp, synthetic construct
  source 1..34: mol_type = other DNA
tcgagctcggtacccaccgaactcctgacagagt

SEQ ID NO: 91 - DNA, 30 bp, synthetic construct
  source 1..30: mol_type = other DNA
acatgaagcgcctcggtacattcttccaca

SEQ ID NO: 92 - DNA, 30 bp, synthetic construct
  source 1..30: mol_type = other DNA
aagaatgtaccgaggcgcttcatgtcaaca

SEQ ID NO: 93 - DNA, 30 bp, synthetic construct
  source 1..30: mol_type = other DNA
caaatgtcttcattgttttgatctcctcca

SEQ ID NO: 94 - DNA, 19 bp, synthetic construct
  source 1..19: mol_type = other DNA
actgcctggtaccaccaga

SEQ ID NO: 95 - DNA, 20 bp, synthetic construct
  source 1..20: mol_type = other DNA
ctgcctctcacaagttgaag

SEQ ID NO: 96 - DNA, 30 bp, synthetic construct
  source 1..30: mol_type = other DNA
tcgagctcggtacccattggtgctcggcgc

SEQ ID NO: 97 - DNA, 29 bp, synthetic construct
  source 1..29: mol_type = other DNA
tgggatgtttctgtgttgttagtctagtg

SEQ ID NO: 98 - DNA, 34 bp, synthetic construct
  source 1..34: mol_type = other DNA
tcgagctcggtacccaaccaagtttagatgcgcc

SEQ ID NO: 99 - DNA, 31 bp, synthetic construct
  source 1..31: mol_type = other DNA
gctgggatgtttctgccgatagtttatgtca

SEQ ID NO: 100 - DNA, 35 bp, synthetic construct
  source 1..35: mol_type = other DNA
tcgagctcggtacccggtgacagctcgcgccgcat

SEQ ID NO: 101 - DNA, 32 bp, synthetic construct
  source 1..32: mol_type = other DNA
gcgctgggatgtttctggcgaaaagttctccc

SEQ ID NO: 102 - DNA, 33 bp, synthetic construct
  source 1..33: mol_type = other DNA
tcgagctcggtacccttgatgcctgcatgaagg

SEQ ID NO: 103 - DNA, 31 bp, synthetic construct
  source 1..31: mol_type = other DNA
tgacatgaagcgccgaatattgatcctatct

SEQ ID NO: 104 - DNA, 33 bp, synthetic construct
  source 1..33: mol_type = other DNA
ttcgagctcggtacccaccttcagcaaccactc

SEQ ID NO: 105 - DNA, 29 bp, synthetic construct
  source 1..29: mol_type = other DNA
tgacatgaagcgccgaaaaattcttctct

SEQ ID NO: 106 - DNA, 32 bp, synthetic construct
  source 1..32: mol_type = other DNA
aaaggaaacactcatgagcaaatatgcagacg

SEQ ID NO: 107 - DNA, 27 bp, synthetic construct
  source 1..27: mol_type = other DNA
ctagaggatcccccagccggagaggga

SEQ ID NO: 108 - DNA, 30 bp, synthetic construct
  source 1..30: mol_type = other DNA
aaaggaaacactcatgaccaaaactgtcgc

SEQ ID NO: 109 - DNA, 31 bp, synthetic construct
  source 1..31: mol_type = other DNA
ctagaggatccccacctctggaggcgtggtc

SEQ ID NO: 110 - DNA, 34 bp, synthetic construct
  source 1..34: mol_type = other DNA
cgaaaggaaacactcatgttgaatgtcactgacc

SEQ ID NO: 111 - DNA, 32 bp, synthetic construct
  source 1..32: mol_type = other DNA
ctagaggatccccccgtgctcagcctgaggag

SEQ ID NO: 112 - DNA, 33 bp, synthetic construct
  source 1..33: mol_type = other DNA
ggagatcaaaacaatgaccttcactattcttcc

SEQ ID NO: 113 - DNA, 32 bp, synthetic construct
  source 1..32: mol_type = other DNA
ctagaggatccccacgaaacgtgcacaacctt

SEQ ID NO: 114 - DNA, 27 bp, synthetic construct
  source 1..27: mol_type = other DNA
gagatcaaaacaatgactgtcgcacca

SEQ ID NO: 115 - DNA, 32 bp, synthetic construct
  source 1..32: mol_type = other DNA
ctagaggatccccgggtcgcggccgtagtggc

SEQ ID NO: 116 - DNA, 32 bp, synthetic construct
  source 1..32: mol_type = other DNA
actagactaacaacacagaaacatcccagcgc

SEQ ID NO: 117 - DNA, 30 bp, synthetic construct
  source 1..30: mol_type = other DNA
tctgcatatttgctcatgagtgtttccttt

SEQ ID NO: 118 - DNA, 33 bp, synthetic construct
  source 1..33: mol_type = other DNA
acataaactatcggcagaaacatcccagcgcta

SEQ ID NO: 119 - DNA, 30 bp, synthetic construct
  source 1..30: mol_type = other DNA
gacagttttggtcatgagtgtttcctttcg

SEQ ID NO: 120 - DNA, 31 bp, synthetic construct
  source 1..31: mol_type = other DNA
gagaacttttcgccagaaacatcccagcgct

SEQ ID NO: 121 - DNA, 30 bp, synthetic construct
  source 1..30: mol_type = other DNA
agtgacattcaacatgagtgtttcctttcg

SEQ ID NO: 122 - DNA, 29 bp, synthetic construct
  source 1..29: mol_type = other DNA
aggatcaatattcggcgcttcatgtcaac

SEQ ID NO: 123 - DNA, 30 bp, synthetic construct
  source 1..30: mol_type = other DNA
gaatagtgaaggtcattgttttgatctcct

SEQ ID NO: 124 - DNA, 29 bp, synthetic construct
  source 1..29: mol_type = other DNA
gagaagaatttttcggcgcttcatgtcaa

SEQ ID NO: 125 - DNA, 29 bp, synthetic construct
  source 1..29: mol_type = other DNA
tggtgcgacagtcattgttttgatctcct

SEQ ID NO: 126 - DNA, 15 bp, synthetic construct
  source 1..15: mol_type = other DNA
gagcatgcatcaaag

SEQ ID NO: 127 - DNA, 19 bp, synthetic construct
  source 1..19: mol_type = other DNA
agaaatttgatccttataa

SEQ ID NO: 128 - DNA, 17 bp, synthetic construct
  source 1..17: mol_type = other DNA
ttgagagatgcttatcg

SEQ ID NO: 129 - DNA, 20 bp, synthetic construct
  source 1..20: mol_type = other DNA
cacttcagtgcggattccaa

SEQ ID NO: 130 - DNA, 17 bp, synthetic construct
  source 1..17: mol_type = other DNA
agcgggtttaattcagg

SEQ ID NO: 131 - DNA, 18 bp, synthetic construct
  source 1..18: mol_type = other DNA
gtgggtaagggttttcgt

SEQ ID NO: 132 - DNA, 19 bp, synthetic construct
  source 1..19: mol_type = other DNA
cacgaaaatgatcgttttg

SEQ ID NO: 133 - DNA, 18 bp, synthetic construct
  source 1..18: mol_type = other DNA
tatgggattcgatggcca

SEQ ID NO: 134 - DNA, 19 bp, synthetic construct
  source 1..19: mol_type = other DNA
tgtgggaatcgctgggcac

SEQ ID NO: 135 - DNA, 16 bp, synthetic construct
  source 1..16: mol_type = other DNA
cggtcgcccgcatctg

SEQ ID NO: 136 - DNA, 31 bp, synthetic construct
  source 1..31: mol_type = other DNA
ttcgagctcggtacccatgaagtctaccggc

SEQ ID NO: 137 - DNA, 30 bp, synthetic construct
  source 1..30: mol_type = other DNA
gacatgaagcgccgacatctaataaccggg

SEQ ID NO: 138 - DNA, 32 bp, synthetic construct
  source 1..32: mol_type = other DNA
ccgacgaggcctaagaactcattccttctgct

SEQ ID NO: 139 - DNA, 31 bp, synthetic construct
  source 1..31: mol_type = other DNA
ctctagaggatccccttagagtgcattgatc

SEQ ID NO: 140 - DNA, 30 bp, synthetic construct
  source 1..30: mol_type = other DNA
ccggttattagatgtcggcgcttcatgtca

SEQ ID NO: 141 - DNA, 25 bp, synthetic construct
  source 1..25: mol_type = other DNA
ggatgtttctctagatgcgggcgat

SEQ ID NO: 142 - DNA, 29 bp, synthetic construct
  source 1..29: mol_type = other DNA
gcccgcatctagagaaacatcccagcgct

SEQ ID NO: 143 - DNA, 29 bp, synthetic construct
  source 1..29: mol_type = other DNA
agaaggaatgagttcttaggcctcgtcgg

SEQ ID NO: 144 - DNA, 19 bp, synthetic construct
  source 1..19: mol_type = other DNA
ctttcagctttccctcccg

SEQ ID NO: 145 - DNA, 17 bp, synthetic construct
  source 1..17: mol_type = other DNA
gctgtacttttagtaca

SEQ ID NO: 146 - DNA, 5802 bp, synthetic construct
  source 1..5802: mol_type = other DNA
gttcgcttgctgtccataaaaccgcccagtctagctatcgccatgtaagcccactgcaagctacctgctttctctttgcgcttgcgttttcccttgtccagatagcccagtagctgacattcatccggggtcagcaccgtttctgcggactggctttctacgtgttccgcttcctttagcagcccttgcgccctgagtgcttgcggcagcgtgaagctagcttttatcgccattcgccattcaggctgcgcaactgttgggaagggcgatcggtgcgggcctcttcgctattacgccagctggcgaaagggggatgtgctgcaaggcgattaagttgggtaacgccagggttttcccagtcacgacgttgtaaaacgacggccagtgaattcgagctcggtacccggggatcctctagagtcgacctgcaggcatgcaagcttggcgtaatcatggtcatagctgtttcctgtgtgaaattgttatccgctcacaattccacacaacatacgagccggaagcataaagtgtaaagcctggggtgcctaatgagtgagctaactcacattaattgcgttgcgctcactgcccgctttccagtcgggaaacctgtcgtgccagctgcattaatgaatcggccaacgcgcggggagaggcggtttgcgtattgggcgctcttccgcttcctcgctcactgactcgctgcgctcggtcgttcggctgcggcgagcggtatcagctcactcaaaggcggtaatacggttatccacagaatcaggggataacgcaggaaagaacatgtgagcaaaaggccagcaaaaggccaggaaccgtaaaaaggccgcgttgctggcgtttttccataggctccgcccccctgacgagcatcacaaaaatcgacgctcaagtcagaggtggcgaaacccgacaggactataaagataccaggcgtttccccctggaagctccctcgtgcgctctcctgttccgaccctgccgcttaccggatacctgtccgcctttctcccttcgggaagcgtggcgctttctcaatgctcacgctgtaggtatctcagttcggtgtaggtcgttcgctccaagctgggctgtgtgcacgaaccccccgttcagcccgaccgctgcgccttatccggtaactatcgtcttgagtccaacccggtaagacacgacttatcgccactggcagcagccactggtaacaggattagcagagcgaggtatgtaggcggtgctacagagttcttgaagtggtggcctaactacggctacactagaaggacagtatttggtatctgcgctctgctgaagccagttaccttcggaaaaagagttggtagctcttgatccggcaaacaaaccaccgctggtagcggtggtttttttgtttgcaagcagcagattacgcgcagaaaaaaaggatctcaagaagatcctttgatcttttctacggggtctgacgctcagtggaacgaaaactcacgttaagggattttggtcatgagattatcaaaaaggatcttcacctagatccttttggggtgggcgaagaactccagcatgagatccccgcgctggaggatcatccagccctgatagaaacagaagccactggagcacctcaaaaacaccatcatacactaaatcagtaagttggcagcatcacccgacgcactttgcgccgaataaatacctgtgacggaagatcacttcgcagaataaataaatcctggtgtccctgttgataccgggaagccctgggccaacttttggcgaaaatgagacgttgatcggcacgtaagaggttccaactttcaccataatgaaataagatcactaccgggcgtattttttgagttatcgagattttcaggagctgatagaaacagaagccactggagcacctcaaaaacaccatcatacactaaatcagtaagttggcagcatcacccgacgcactttgcgccgaataaatacctgtgacggaagatcacttcgcagaataaataaatcctggtgtccctgttgataccgggaagccctgggccaacttttggcgaaaatgagacgttgatcggcacgtaagaggttccaactttcaccataatgaaataagatcactaccgggcgtattttttgagttatcgagattttcaggagctctttggcatcgtctctcgcctgtcccctcagttcagtaatttcctgcatttgcctgtttccagtcggtagatattccacaaaacagcagggaagcagcgcttttccgctgcataaccctgcttcggggtcattatagcgattttttcggtatatccatcctttttcgcacgatatacaggattttgccaaagggttcgtgtagactttccttggtgtatccaacggcgtcagccgggcaggataggtgaagtaggcccacccgcgagcgggtgttccttcttcactgtcccttattcgcacctggcggtgctcaacgggaatcctgctctgcgaggctggccggctaccgccggcgtaacagatgagggcaagcggatggctgatgaaaccaagccaaccaggaagggcagcccacctatcaaggtgtactgccttccagacgaacgaagagcgattgaggaaaaggcggcggcggccggcatgagcctgtcggcctacctgctggccgtcggccagggctacaaaatcacgggcgtcgtggactatgagcacgtccgcgagggcgtcccggaaaacgattccgaagcccaacctttcatagaaggcggcggtggaatcgaaatctcgtgatggcaggttgggcgtcgcttggtcggtcatttcgaaaaaggttaggaatacggttagccatttgcctgcttttatatagttcatatgggattcacctttatgttgataagaaataaaagaaaatgccaataggatatcggcattttcttttgcgtttttatttgttaactgttaattgtccttgttcaaggatgctgtctttgacaacagatgttttcttgcctttgatgttcagcaggaagctcggcgcaaacgttgattgtttgtctgcgtagaatcctctgtttgtcatatagcttgtaatcacgacattgtttcctttcgcttgaggtacagcgaagtgtgagtaagtaaaggttacatcgttaggcggatcaagatccatttttaacacaaggccagttttgttcagcggcttgtatgggccagttaaagaattagaaacataaccaagcatgtaaatatcgttagacgtaatgccgtcaatcgtcatttttgatccgcgggagtcagtgaacaggtaccatttgccgttcattttaaagacgttcgcgcgttcaatttcatctgttactgtgttagatgcaatcagcggtttcatcacttttttcagtgtgtaatcatcgtttagctcaatcataccgagagcgccgtttgctaactcagccgtgcgttttttatcgctttgcagaagtttttgactttcttgacggaagaatgatgtgcttttgccatagtatgctttgttaaataaagattcttcgccttggtagccatcttcagttccagtgtttgcttcaaatactaagtatttgtggcctttatcttctacgtagtgaggatctctcagcgtatggttgtcgcctgagctgtagttgccttcatcgatgaactgctgtacattttgatacgtttttccgtcaccgtcaaagattgatttataatcctctacaccgttgatgttcaaagagctgtctgatgctgatacgttaacttgtgcagttgtcagtgtttgtttgccgtaatgtttaccggagaaatcagtgtagaataaacggatttttccgtcagatgtaaatgtggctgaacctgaccattcttgtgtttggtcttttaggatagaatcatttgcatcgaatttgtcgctgtctttaaagacgcggccagcgtttttccagctgtcaatagaagtttcgccgactttttgatagaacatgtaaatcgatgtgtcatccgcatttttaggatctccggctaatgcaaagacgatgtggtagccgtgatagtttgcgacagtgccgtcagcgttttgtaatggccagctgtcccaaacgtccaggccttttgcagaagagatatttttaattgtggacgaatcaaattcagaaacttgatatttttcatttttttgctgttcagggatttgcagcatatcatggcgtgtaatatgggaaatgccgtatgtttccttatatggcttttggttcgtttctttcgcaaacgcttgagttgcgcctcctgccagcagtgcggtagtaaaggttaatactgttgcttgttttgcaaactttttgatgttcatcgttcatgtctccttttttatgtactgtgttagcggtctgcttcttccagccctcctgtttgaagatggcaagttagttacgcacaataaaaaaagacctaaaatatgtaaggggtgacgccaaagtatacactttgccctttacacattttaggtcttgcctgctttatcagtaacaaacccgcgcgatttacttttcgacctcattctattagactctcgtttggattgcaactggtctattttcctcttttgtttgatagaaaatcataaaaggatttgcagactacgggcctaaagaactaaaaaatctatctgtttcttttcattctctgtattttttatagtttctgttgcatgggcataaagttgcctttttaatcacaattcagaaaatatcataatatctcatttcactaaataatagtgaacggcaggtatatgtgatgggttaaaaaggatcaccccagagtcccgctcagaagaactcgtcaagaaggcgatagaaggcgatgcgctgcgaatcgggagcggcgataccgtaaagcacgaggaagcggtcagcccattcgccgccaagctcttcagcaatatcacgggtagccaacgctatgtcctgatagcggtccgccacacccagccggccacagtcgatgaatccagaaaagcggccattttccaccatgatattcggcaagcaggcatcgccatgggtcacgacgagatcctcgccgtcgggcatccgcgccttgagcctggcgaacagttcggctggcgcgagcccctgatgctcttcgtccagatcatcctgatcgacaagaccggcttccatccgagtacgtgctcgctcgatgcgatgtttcgcttggtggtcgaatgggcaggtagccggatcaagcgtatgcagccgccgcattgcatcagccatgatggatactttctcggcaggagcaaggtgagatgacaggagatcctgccccggcacttcgcccaatagcagccagtcccttcccgcttcagtgacaacgtcgagacagctgcgcaaggaacgcccgtcgtggccagccacgatagccgcgctgcctcgtcttggagttcattcagggcaccggacaggtcggtcttgacaaaaagaaccgggcgcccctgcgctgacagccggaacacggcggcatcagagcagccgattgtctgttgtgcccagtcatagccgaatagcctctccacccaagcggccggagaacctgcgtgcaatccatcttgttcaatcatgcgaaacgatcctcatcctgtctcttgatcagatcttgatcccctgcgccatcagatccttggcggcaagaaagccatccagtttactttgcagggcttcccaaccttaccagagggcgccccagctggcaattccg